European Patent Application EP 4 481 036 A1, published December 25, 2024. Title: Method for generating human pluripotent stem cell-derived Leydig-like cells and human pluripotent stem cell-derived Leydig-like cell population. Applicant: NATIONAL UNIVERSITY CORPORATION KOBE UNIVERSITY. The sequence listing filed with the application follows.

SEQUENCE LISTING (2 sequences)

SEQ ID NO: 1 - DNA, 3074 bp, Homo sapiens
  source 1..3074: mol_type = genomic DNA
  CDS 167..1552: protein_id = 2; translation = MDYSYDEDLDELCPVCGDKVSGYHYGLLTCESCKGFFKRTVQNNKHYTCTESQSCKIDKTQRKRCPFCRFQKCLTVGMRLEAVRADRMRGGRNKFGPMYKRDRALKQQKKAQIRANGFKLETGPPMGVPPPPPPAPDYVLPPSLHGPEPKGLAAGPPAGPLGDFGAPALPMAVPGAHGPLAGYLYPAFPGRAIKSEYPEPYASPPQPGLPYGYPEPFSGGPNVPELILQLLQLEPDEDQVRARILGCLQEPTKSRPDQPAAFGLLCRMADQTFISIVDWARRCMVFKELEVADQMTLLQNCWSELLVFDHIYRQVQHGKEGSILLVTGQEVELTTVATQAGSLLHSLVLRAQELVLQLLALQLDRQEFVCLKFIILFSLDLKFLNNHILVKDAQEKANAALLDYTLCHYPHCGDKFQQLLLCLVEVRALSMQAKEYLYHKHLGNEMPRNNLLIEMLQAKQT
agcctgctgtccggctgccgcccgccgtggtgtgagggggtttctgcgcacccacagtcgccaccgtcccacctgggctgccggagcctccccctggacccctggtgcccactgccaccctcatccggtgtgagagcgctgcttccgcttcgcggacgccgcgggcatggactattcgtacgacgaggacctggacgagctgtgccccgtgtgcggggacaaggtgtccggctaccactacggactgctcacgtgtgagagctgcaagggcttcttcaagcgcacggtgcagaacaacaagcactacacgtgcaccgagagccagagctgcaagatcgacaagacgcagcgcaagcgctgtcccttctgccgcttccagaaatgcctgacggtggggatgcgcctggaagccgtgcgcgctgaccgtatgaggggtggccggaacaagtttgggccgatgtacaagcgggaccgggccctgaaacagcagaagaaggcacagattcgggccaatggcttcaagctggagacagggcccccgatgggggtgcccccgccgccccctcccgcaccggactacgtgctgcctcccagcctgcatgggcctgagcccaagggcctggccgccggtccacctgctgggccactgggcgactttggggccccagcactgcccatggccgtgcccggtgcccacgggccactggctggctacctctaccctgcctttcctggccgtgccatcaagtctgagtacccggagccttatgccagccccccacagcctgggctgccgtacggctacccagagcccttctctggagggcccaacgtgcctgagctcatcctgcagctgctgcagctggagccggatgaggaccaggtgcgggcccgcatcttgggctgcctgcaggagcccaccaaaagccgccccgaccagccggcggccttcggcctcctgtgcagaatggccgaccagaccttcatctccatcgtggactgggcacgcaggtgcatggtcttcaaggagctggaggtggccgaccagatgacgctgctgcagaactgctggagcgagctgctggtgttcgaccacatctaccgccaggtccagcacggcaaggagggcagcatcctgctggtcaccgggcaggaggtggagctgaccacagtggccacccaggcgggctcgctgctgcacagcctggtgttgcgggcgcaggagctggtgctgcagctgcttgcgctgcagctggaccggcaggagtttgtctgcctcaagttcatcatcctcttcagcctggatttgaagttcctgaataaccacatcctggtgaaagacgctcaggagaaggccaacgccgccctgcttgactacaccctgtgccactacccgcactgcggggacaaattccagcagctgctgctgtgcctggtggaggtgcgggccctgagcatgcaggccaaggagtacctgtaccacaagcacctgggcaacgagatgccccgcaacaacctgctcatcgaaatgctgcaagccaagcagacttgagcctgggccgggggcggggccgggactgggggcgggactgggggcggggcctgggcggggccgcagccacaccgctggctccgcatggttcattttctgatgcccaccgaggagccccagccccgtcccagaggccgctgcccctgagttctgacactgtgtgtttgggaaggtgggtgaggctgggcagggcctggcggaggtggagtggccactggcacttgcctgctgcttggagtgccccaaggaggtggctgttaaccacccgccccgccccctccctgctcccagctctctctcctggagtctgaagcctgcaggtccggggaggaggttcgggattccctggtgggcctcgacgtcccttggatcagaggtcatcccttcctcctctcctggaaacagacagggagaagttgagcaggtatcaactaggggaggagagagggtctccagtgttccccccatagagaccaggagggagagcctctgttttgtaaactaaggataaccgagtttgctaaattgagaggggctattgggccctagaggacactaggagactggttaggacaaaaagaccttctccctagcccttctaccccacctgacctctgcaagagggggcattgatacatcatcgggaaaaaactttgctccaggcatcactgattccctctcccacccaaggagaacgtttggtacaatcgacatcctagccccacccagaggtggccctcccaggctggtatttatctgcaaggttgtagtcaagaggtttttctccccgctttttgtttttaagcttctagacactccttgaaatgtgtgtgtgatggagggaaggggacagatttgaggactgaagctggggcttggggattgccactaagtacagctgacggtttctccccggacactcgcctactaagtacccttggggtggtgctgggtcattacttctgagccccagccccaatccagagaagcgctgttgcccgccctccacccactaggtgaacagcaggatgccctgttgggggcttcaggtctctgtgggtgggaatgcaagtgaacttgggagggggcacgggcctgtagatcagggatagcgctgttgatcccctctctgtggctccaacccgttgggtcccttgctgcaaacccatgaagctggccctcagctccctgaccccctgtcctaggtcatgaaggacactctgcagggtgaagcaccagggagaggcctcggctgtctcctgtccccggcggggtgcctgctgtccgtcccgctttcatgttactgttgcagcttgtgctgagcctgcccagttggaggagactgggcacccctgcctcctgcctcccgcctcccgccaccctgtctcagtacctcccctccccgccccctgaaacatgtgcccctgccaaggccggagacccacagccctgaaacgagaagtgcccttaaggatcaccccagcccccacagccctggaataaatttcgcaattagtttcca

SEQ ID NO: 2 - protein, 461 aa, Homo sapiens
MDYSYDEDLDELCPVCGDKVSGYHYGLLTCESCKGFFKRTVQNNKHYTCTESQSCKIDKTQRKRCPFCRFQKCLTVGMRLEAVRADRMRGGRNKFGPMYKRDRALKQQKKAQIRANGFKLETGPPMGVPPPPPPAPDYVLPPSLHGPEPKGLAAGPPAGPLGDFGAPALPMAVPGAHGPLAGYLYPAFPGRAIKSEYPEPYASPPQPGLPYGYPEPFSGGPNVPELILQLLQLEPDEDQVRARILGCLQEPTKSRPDQPAAFGLLCRMADQTFISIVDWARRCMVFKELEVADQMTLLQNCWSELLVFDHIYRQVQHGKEGSILLVTGQEVELTTVATQAGSLLHSLVLRAQELVLQLLALQLDRQEFVCLKFIILFSLDLKFLNNHILVKDAQEKANAALLDYTLCHYPHCGDKFQQLLLCLVEVRALSMQAKEYLYHKHLGNEMPRNNLLIEMLQAKQT